European Patent Specification EP 3 524 689 B1, published September 6, 2023. Title: METHODS FOR PREDICTING THE PROGNOSIS OF BREAST CANCER PATIENT. Applicant: Gencurix Inc. Application 17874456.1. The sequence listing filed with the application follows.

SEQUENCE LISTING (27 sequences)

SEQ ID NO: 1 - DNA, 19 bp, Artificial Sequence
  UBE2C forward primer
aaaaggctacagcaggagc

SEQ ID NO: 2 - DNA, 19 bp, Artificial Sequence
  UBE2C reverse primer
agctgctccatggatggtc

SEQ ID NO: 3 - DNA, 24 bp, Artificial Sequence
  TOP2A forward primer
aagagtcattccacgaataaccat

SEQ ID NO: 4 - DNA, 20 bp, Artificial Sequence
  TOP2A reverse primer
gagggcttccttcagtattt

SEQ ID NO: 5 - DNA, 18 bp, Artificial Sequence
  RRM2 forward primer
tgggaatccctgaaaccc

SEQ ID NO: 6 - DNA, 19 bp, Artificial Sequence
  RRM2 reverse primer
gaacttcttggctaaatcg

SEQ ID NO: 7 - DNA, 21 bp, Artificial Sequence
  FOXM1 forward primer
aagcacattgccaagccaggc

SEQ ID NO: 8 - DNA, 19 bp, Artificial Sequence
  FOXM1 reverse primer
cagggaaaggttgtggcgg

SEQ ID NO: 9 - DNA, 21 bp, Artificial Sequence
  MKI67 forward primer
cagaatgagagctcccagcct

SEQ ID NO: 10 - DNA, 21 bp, Artificial Sequence
  MKI67 reverse primer
tgcatgagaaccttcgcactc

SEQ ID NO: 11 - DNA, 18 bp, Artificial Sequence
  BTN3A2 forward primer
cttcaagcctggtgagga

SEQ ID NO: 12 - DNA, 21 bp, Artificial Sequence
  BTN3A2 reverse primer
ttttctgcagtctatttttcc

SEQ ID NO: 13 - DNA, 17 bp, Artificial Sequence
  CTBP1 forward primer
ccttgggcatcatcgga

SEQ ID NO: 14 - DNA, 18 bp, Artificial Sequence
  CTBP1 reverse primer
gttgaagccgaaggcctt

SEQ ID NO: 15 - DNA, 22 bp, Artificial Sequence
  CUL1 forward primer
agtactgaattcttgcagcaga

SEQ ID NO: 16 - DNA, 23 bp, Artificial Sequence
  CUL1 reverse primer
tcttcgttgttcctcaagcagac

SEQ ID NO: 17 - DNA, 22 bp, Artificial Sequence
  UBQLN1 forward primer
gaaatcctcagcttcaagaaca

SEQ ID NO: 18 - DNA, 22 bp, Artificial Sequence
  UBQLN1 reverse primer
tgacattgctgatagtgtatca

SEQ ID NO: 19 - DNA, 8 bp, Artificial Sequence
  UBE2C UPL probe
gggaaggc

SEQ ID NO: 20 - DNA, 8 bp, Artificial Sequence
  TOP2A UPL probe
gcctctga

SEQ ID NO: 21 - DNA, 8 bp, Artificial Sequence
  RRM2 UPL probe
aaagccag

SEQ ID NO: 22 - DNA, 8 bp, Artificial Sequence
  FOXM1 UPL probe
aggctgga

SEQ ID NO: 23 - DNA, 8 bp, Artificial Sequence
  MKI67 UPL probe
gaggagag

SEQ ID NO: 24 - DNA, 8 bp, Artificial Sequence
  BTN3A2 UPL probe
caaggtgg

SEQ ID NO: 25 - DNA, 8 bp, Artificial Sequence
  CTBP1 UPL probe
gccccacg

SEQ ID NO: 26 - DNA, 8 bp, Artificial Sequence
  CUL1 UPL probe
gcagaggc

SEQ ID NO: 27 - DNA, 8 bp, Artificial Sequence
  UBQLN1 UPL probe
ttgggagc